European Patent Specification EP 3 157 570 B1, published June 7, 2023. Title: Peptide-based compounds and their uses for tumor imaging and targeting. Applicant: Klinikum rechts der Isar der TU München Helmholtz Zentrum München. The sequence listing filed with the application follows.

SEQUENCE LISTING (4 sequences)

SEQ ID NO: 1 - protein, 14 aa, Artificial Sequence
  TPP peptide wherein Xaa is Ser or Thr
  misc_feature (13)..(13): Xaa can be any naturally occurring amino acid
TKDNNLLGRFELXG

SEQ ID NO: 2 - protein, 14 aa, Homo sapiens
TKDNNLLGRFELSG

SEQ ID NO: 3 - protein, 14 aa, Homo sapiens
TKDNNLLGRFELTG

SEQ ID NO: 4 - protein, 14 aa, Artificial Sequence
  scrambled control peptide
NGLTLKNDFSRLEG